European Patent Specification EP 3 492 606 B1, published October 4, 2023. Title: Urine Biomarkers. Applicant: Exosome Diagnostics, Inc. Russo, Leileata M. Application PCT/US2012/051918. The sequence listing filed with the application follows.

SEQUENCE LISTING (3 sequences)

SEQ ID NO: 1 - DNA, 16 bp, Artificial Sequence
  Synthesized primer
ctgcacgcgctggctc

SEQ ID NO: 2 - DNA, 20 bp, Artificial Sequence
  Synthesized primer
tcttcatctgctggtcggaa

SEQ ID NO: 3 - DNA, 21 bp, Artificial Sequence
  Synthesized primer
caaattctcaccagtccgtct